European Patent Specification EP 3 528 837 B1, published June 10, 2026. Title: New antimicrobial agents against Enterococcus bacteria. Applicant: Lysando AG. The sequence listing filed with the application follows.

SEQUENCE LISTING (105 sequences)

SEQ ID NO: 1 - protein, 314 aa, Enterococcal bacteriophage phi1
MSNINMETAIANMYALKARGITYSMNYSRTGADGTGDCSGTVYDSLRKAGASDAGWVLNTDSMHSWLEKNGFKLIAQNKEWSAKRGDVVIFGKKGASGGSAGHVVIFISSTQIIHCTWKSATANGVYVDNEATTCPYSMGWYVYRLNGGSTPPKPNTKKVKVLKHATNWSPSSKGAKMASFVKGGTFEVKQQRPISYSYSNQEYLIVNKGTVLGWVLSQDIEGGYGSDRVGGSKPKLPAGFTKEEATFINGNAPITTRKNKPSLSSQTATPLYPGQSVRYLGWKSAEGYIWIYATDGRYIPVRPVGKEAWGTFK

SEQ ID NO: 2 - protein, 150 aa, Enterococcal bacteriophage phi1
INMETAIANMYALKARGITYSMNYSRTGADGTGDCSGTVYDSLRKAGASDAGWVLNTDSMHSWLEKNGFKLIAQNKEWSAKRGDVVIFGKKGASGGSAGHVVIFISSTQIIHCTWKSATANGVYVDNEATTCPYSMGWYVYRLNGGSTPP

SEQ ID NO: 3 - protein, 65 aa, Enterococcal bacteriophage phi1
EATFINGNAPITTRKNKPSLSSQTATPLYPGQSVRYLGWKSAEGYIWIYATDGRYIPVRPVGKEA

SEQ ID NO: 4 - protein, 21 aa, unknown
  Buforin II vertebrate
TRSSRAGLQFPVGRVHRLLRK

SEQ ID NO: 5 - protein, 313 aa, Enterococcal bacteriophage phi1
SNINMETAIANMYALKARGITYSMNYSRTGADGTGDCSGTVYDSLRKAGASDAGWVLNTDSMHSWLEKNGFKLIAQNKEWSAKRGDVVIFGKKGASGGSAGHVVIFISSTQIIHCTWKSATANGVYVDNEATTCPYSMGWYVYRLNGGSTPPKPNTKKVKVLKHATNWSPSSKGAKMASFVKGGTFEVKQQRPISYSYSNQEYLIVNKGTVLGWVLSQDIEGGYGSDRVGGSKPKLPAGFTKEEATFINGNAPITTRKNKPSLSSQTATPLYPGQSVRYLGWKSAEGYIWIYATDGRYIPVRPVGKEAWGTFK

SEQ ID NO: 6 - protein, 6 aa, artificial
  synthetic sequence
KRKKRK

SEQ ID NO: 7 - protein, 5 aa, artificial
  synethtic sequence
  misc_feature (3)..(3): Xaa can be any naturally occurring amino acid
KRXKR

SEQ ID NO: 8 - protein, 5 aa, artificial
  synthetic sequence
KRSKR

SEQ ID NO: 9 - protein, 5 aa, artificial
  synthetic sequence
KRGSG

SEQ ID NO: 10 - protein, 9 aa, artificial
  synthetic sequence
KRKKRKKRK

SEQ ID NO: 11 - protein, 9 aa, artificial
  synthetic sequence
RRRRRRRRR

SEQ ID NO: 12 - protein, 8 aa, artificial
  synthetic sequence
KKKKKKKK

SEQ ID NO: 13 - protein, 10 aa, artificial
  synthetic sequence
KRKKRKKRKK

SEQ ID NO: 14 - protein, 12 aa, artificial
  synthetic sequence
KRKKRKKRKKRK

SEQ ID NO: 15 - protein, 14 aa, artificial
  synthetic sequence
KRKKRKKRKKRKKR

SEQ ID NO: 16 - protein, 16 aa, artificial
  synthetic sequence
KKKKKKKKKKKKKKKK

SEQ ID NO: 17 - protein, 18 aa, artificial
  synthetic sequence
KRKKRKKRKKRKKRKKRK

SEQ ID NO: 18 - protein, 19 aa, artificial
  synthetic sequence
KRKKRKKRKKRKKRKKRKK

SEQ ID NO: 19 - protein, 19 aa, artificial
  synthetic sequence
RRRRRRRRRRRRRRRRRRR

SEQ ID NO: 20 - protein, 19 aa, artificial
  synthetic sequence
KKKKKKKKKKKKKKKKKKK

SEQ ID NO: 21 - protein, 20 aa, artificial
  synthetic sequence
KRKKRKKRKRSKRKKRKKRK

SEQ ID NO: 22 - protein, 21 aa, artificial
  synthetic sequence
KRKKRKKRKRSKRKKRKKRKK

SEQ ID NO: 23 - protein, 21 aa, artificial
  synthetic sequence
KRKKRKKRKKRKKRKKRKKRK

SEQ ID NO: 24 - protein, 22 aa, artificial
  synthetic sequence
KRKKRKKRKRGSGKRKKRKKRK

SEQ ID NO: 25 - protein, 24 aa, artificial
  synthetic sequence
KRKKRKKRKRGSGSGKRKKRKKRK

SEQ ID NO: 26 - protein, 25 aa, artificial
  synthetic sequence
KRKKRKKRKKRKKRKKRKKRKKRKK

SEQ ID NO: 27 - protein, 31 aa, artificial
  synthetic sequence
KRKKRKKRKRSKRKKRKKRKRSKRKKRKKRK

SEQ ID NO: 28 - protein, 38 aa, artificial
  synthetic sequence
KRKKRKKRKRGSGSGKRKKRKKRKGSGSGKRKKRKKRK

SEQ ID NO: 29 - protein, 39 aa, artificial
  synthetic sequence
KRKKRKKRKKRKKRKKRKKRKKRKKRKKRKKRKKRKKRK

SEQ ID NO: 30 - protein, 42 aa, artificial
  synthetic sequence
KRKKRKKRKRSKRKKRKKRKRSKRKKRKKRKRSKRKKRKKRK

SEQ ID NO: 31 - protein, 37 aa, Homo sapiens
LLGDFFRKSKEKIGKEFKRIVQRIKDFLRNLVPRTES

SEQ ID NO: 32 - protein, 29 aa, unknown
  SMAP-29 sheep
RGLRRLGRKIAHGVKKYGPTVLRIIRIAG

SEQ ID NO: 33 - protein, 13 aa, unknown
  Indolicidine bovine
ILPWKWPWWPWRR

SEQ ID NO: 34 - protein, 18 aa, unknown
  Protegrin Porcine
RGGRLCYCRRRFCVCVGR

SEQ ID NO: 35 - protein, 31 aa, unknown
  Cecropin P1 Mammal (pig)
SWLSKTAKKLENSAKKRISEGIAIAIQGGPR

SEQ ID NO: 36 - protein, 23 aa, unknown
  Magainin frog
GIGKFLHSAKKFGKAFVGEIMNS

SEQ ID NO: 37 - protein, 25 aa, unknown
  Pleurocidin fish
GWGSFFKKAAHVGKHVGKAALTHYL

SEQ ID NO: 38 - protein, 36 aa, Aedes aegypti
GGLKKLGKKLEGAGKRVFNAAEKALPVVAGAKALRK

SEQ ID NO: 39 - protein, 40 aa, Drosophila melanogaster
GWLKKIGKKIERVGQHTRDATIQGLGIPQQAANVAATARG

SEQ ID NO: 40 - protein, 39 aa, unknown
  Sarcotoxin IA Fly
GWLKKIGKKIERVGQHTRDATIQGLGIAQQAANVAATAR

SEQ ID NO: 41 - protein, 17 aa, Apis mellifera
ANRPVYIPPPRPPHPRL

SEQ ID NO: 42 - protein, 24 aa, unknown
  Ascaphine 5 Frog
GIKDWIKGAAKKLIKTVASHIANQ

SEQ ID NO: 43 - protein, 22 aa, unknown
  Nigrocine 2 Frog
GLLSKVLGVGKKVLCGVSGLVC

SEQ ID NO: 44 - protein, 24 aa, unknown
  Pseudin 1 Rana Frog
GLNTLKKVFQGLHEAIKLINNHVQ

SEQ ID NO: 45 - protein, 18 aa, unknown
  Ranalexin Frog
FLGGLIVPAMICAVTKKC

SEQ ID NO: 46 - protein, 26 aa, unknown
  Melittin bee
GIGAVLKVLTTGLPALISWIKRKRQQ

SEQ ID NO: 47 - protein, 25 aa, unknown
  Lycotoxin 1 Spider
IWLTALKFLGKHAAKKLAKQQLSKL

SEQ ID NO: 48 - protein, 19 aa, unknown
  Parasin 1 Fish
KGRGKQGGKVRAKAKTRSS

SEQ ID NO: 49 - protein, 39 aa, unknown
  Buforin I Toad
AGRGKQGGKVRAKAKTRSSRAGLQFPVGRVHRLLRKGNY

SEQ ID NO: 50 - protein, 34 aa, unknown
  Dermaseptin 1 Frog
ALWKTMLKKLGTMALHAGKAALGAAADTISQGTQ

SEQ ID NO: 51 - protein, 12 aa, unknown
  Bactenecin 1 Cow
RLCRIVVIRVCR

SEQ ID NO: 52 - protein, 21 aa, unknown
  Thanatin Insect
GSKKPVPIIYCNRRTGKCQRM

SEQ ID NO: 53 - protein, 19 aa, unknown
  Brevinin 1T Rana frogs
VNPIILGVLPKVCLITKKC

SEQ ID NO: 54 - protein, 26 aa, unknown
  Ranateurin 1 Rana frog
SMLSVLKNLGKVGLGFVACKINIKQC

SEQ ID NO: 55 - protein, 46 aa, unknown
  Esculentin 1 Rana frogs
GIFSKLGRKKIKNLLISGLKNVGKEVGMDVVRTGIKIAGCKIKGEC

SEQ ID NO: 56 - protein, 17 aa, Limulus polyphemus
RWCFRVCYRGICYRKCR

SEQ ID NO: 57 - protein, 25 aa, unknown
  Androctonin Scorpion
RSVCRQIKICRRRGGCYYKCTNRPY

SEQ ID NO: 58 - protein, 30 aa, Homo sapiens
DCYCRIPACIAGERRYGTCIYQGRLWAFCC

SEQ ID NO: 59 - protein, 38 aa, unknown
  beta-defensin cow
NPVSCVRNKGICVPIRCPGSMKQIGTCVGRAVKCCRKK

SEQ ID NO: 60 - protein, 18 aa, unknown
  theta-defensin monkey
GFCRCLCRRGVCRCICTR

SEQ ID NO: 61 - protein, 40 aa, unknown
  defensin (sapecin A) insect
ATCDLLSGTGINHSACAAHCLLRGNRGGYCNGKAVCVCRN

SEQ ID NO: 62 - protein, 46 aa, unknown
  Thionin (crambin) plant
TTCCPSIVARSNFNVCRIPGTPEAICATYTGCIIIPGATCPGDYAN

SEQ ID NO: 63 - protein, 50 aa, unknown
  defensin from radish
QKLCQRPSGTWSGVCGNNNACKNQCIRLEKARHGSCNYVFPAHCICYFPC

SEQ ID NO: 64 - protein, 44 aa, Drosophila melanogaster
DCLSGRYKGPCAVWDNETCRRVCKEEGRSSGHCSPSLKCWCEGC

SEQ ID NO: 65 - protein, 25 aa, Homo sapiens
DTHFPICIFCCGCCHRSKCGMCCKT

SEQ ID NO: 66 - protein, 44 aa, unknown
  Bac 5 Cow
RFRPPIRRPPIRPPFYPPFRPPIRPPIFPPIRPPFRPPLGRPFP

SEQ ID NO: 67 - protein, 39 aa, unknown
  PR-39 Pig
RRRPRPPYLPRPRPPPFFPPRLPPRIPPGFPPRFPPRFP

SEQ ID NO: 68 - protein, 20 aa, unknown
  Pyrrhocoricin Insect
VDKGSYLPRPTPPRPIYNRN

SEQ ID NO: 69 - protein, 24 aa, Homo sapiens
DSHAKRHHGYKRKFHEKHHSHRGY

SEQ ID NO: 70 - protein, 19 aa, Unknown
  ECP19
RPPQFTRAQWFAIQHISLN

SEQ ID NO: 71 - protein, 23 aa, Unknown
  MSI-594
GIGKFLKKAKKGIGAVLKVLTTG

SEQ ID NO: 72 - protein, 35 aa, Unknown
  TL-ColM
METLTVHAPSPSTNLPSYGNGAFSLSAPHVPGAGP

SEQ ID NO: 73 - protein, 18 aa, Unknown
  SBO
KLKKIAQKIKNFFAKLVA

SEQ ID NO: 74 - protein, 26 aa, unknown
  Macedocin
GKNGVFKTISHECHLNTWAFLATCCS

SEQ ID NO: 75 - protein, 22 aa, unknown
  Macedocin (Trunc)
GKNGVFKTISHECHLNTWAFLA

SEQ ID NO: 76 - protein, 28 aa, unknown
  D16
ACKLKSLLKTLSKAKKKKLKTLLKALSK

SEQ ID NO: 77 - protein, 17 aa, unknown
  CPF-C1
GFGSLLGKALRLGANVL

SEQ ID NO: 78 - protein, 34 aa, unknown
  TL-ColM
ETLTVHAPSPSTNLPSYGNGAFSLSAPHVPGAGP

SEQ ID NO: 79 - protein, 26 aa, unknown
  TM-174E
LISKGWPYLLVVVLGATIYFWGNSNG

SEQ ID NO: 80 - protein, 45 aa, unknown
  ECP45
RPPQFTRAQWFAIQHISLNPPRCTIAMRAINNYRWRCKNQNTFLR

SEQ ID NO: 81 - protein, 50 aa, unknown
  ColicinE3_1-51 (S37F)
SGGDGRGHNTGAHSTSGNINGGPTGLGVGGGASDGFGWSSENNPWGGGSG

SEQ ID NO: 82 - protein, 68 aa, unknown
  ColicinE3_1-69 (S37F)
SGGDGRGHNTGAHSTSGNINGGPTGLGVGGGASDGFGWSSENNPWGGGSGSGIHWGGGSGHGNGGGNG

SEQ ID NO: 83 - protein, 52 aa, unknown
  ColicinD_1-53
SDYEGSGPTEGIDYGHSMVVWPSTGLISGGDVKPGGSSGIAPSMPPGWGDYS

SEQ ID NO: 84 - protein, 34 aa, Limulus polyphemus
GFKLKGMARISCLPNGQWSNFPPKCIRECAMVSS

SEQ ID NO: 85 - protein, 18 aa, artificial
  synthetic sequence
GFFIPAVILPSIAFLIVP

SEQ ID NO: 86 - protein, 5 aa, artificial
  synthetic sequence
FFVAP

SEQ ID NO: 87 - protein, 13 aa, unknown
  alpha4-helix of T4 lysozyme
PNRAKRVITTFRT

SEQ ID NO: 88 - protein, 27 aa, artificial
  synthetic sequence
KRWVKRVKRVKRWVKRVVRVVKRWVKR

SEQ ID NO: 89 - protein, 25 aa, Artificial Sequence
  synthetic sequence; MW2
GKPGWLIKVALKFKKLIRRPLKRLA

SEQ ID NO: 90 - protein, 5 aa, Artificial
  Linker sequence
GGGGS

SEQ ID NO: 91 - protein, 6 aa, artificial sequence
  His-Tag (6x)
HHHHHH

SEQ ID NO: 92 - protein, 336 aa, Artificial sequence
  Enterococcal bacteriophae phi1 endolysin plus Buforin II, w/o starting methionine
TRSSRAGLQFPVGRVHRLLRKGSSNINMETAIANMYALKARGITYSMNYSRTGADGTGDCSGTVYDSLRKAGASDAGWVLNTDSMHSWLEKNGFKLIAQNKEWSAKRGDVVIFGKKGASGGSAGHVVIFISSTQIIHCTWKSATANGVYVDNEATTCPYSMGWYVYRLNGGSTPPKPNTKKVKVLKHATNWSPSSKGAKMASFVKGGTFEVKQQRPISYSYSNQEYLIVNKGTVLGWVLSQDIEGGYGSDRVGGSKPKLPAGFTKEEATFINGNAPITTRKNKPSLSSQTATPLYPGQSVRYLGWKSAEGYIWIYATDGRYIPVRPVGKEAWGTFK

SEQ ID NO: 93 - protein, 337 aa, Artificial sequence
  Enterococcal bacteriophae phi1 endolysin plus Buforin II
MTRSSRAGLQFPVGRVHRLLRKGSSNINMETAIANMYALKARGITYSMNYSRTGADGTGDCSGTVYDSLRKAGASDAGWVLNTDSMHSWLEKNGFKLIAQNKEWSAKRGDVVIFGKKGASGGSAGHVVIFISSTQIIHCTWKSATANGVYVDNEATTCPYSMGWYVYRLNGGSTPPKPNTKKVKVLKHATNWSPSSKGAKMASFVKGGTFEVKQQRPISYSYSNQEYLIVNKGTVLGWVLSQDIEGGYGSDRVGGSKPKLPAGFTKEEATFINGNAPITTRKNKPSLSSQTATPLYPGQSVRYLGWKSAEGYIWIYATDGRYIPVRPVGKEAWGTFK

SEQ ID NO: 94 - protein, 345 aa, Artificial sequence
  Enterococcal bacteriophae phi1 endolysin plus Buforin II and HisTag
MTRSSRAGLQFPVGRVHRLLRKGSSNINMETAIANMYALKARGITYSMNYSRTGADGTGDCSGTVYDSLRKAGASDAGWVLNTDSMHSWLEKNGFKLIAQNKEWSAKRGDVVIFGKKGASGGSAGHVVIFISSTQIIHCTWKSATANGVYVDNEATTCPYSMGWYVYRLNGGSTPPKPNTKKVKVLKHATNWSPSSKGAKMASFVKGGTFEVKQQRPISYSYSNQEYLIVNKGTVLGWVLSQDIEGGYGSDRVGGSKPKLPAGFTKEEATFINGNAPITTRKNKPSLSSQTATPLYPGQSVRYLGWKSAEGYIWIYATDGRYIPVRPVGKEAWGTFKLEHHHHHH

SEQ ID NO: 95 - DNA, 450 bp, Artificial sequence
  encoding SEQ ID NO2
atcaatatggaaaccgccattgcaaatatgtatgcactgaaagcacgtggcattacctatagcatgaattatagccgtaccggtgcagatggcaccggtgattgtagcggcaccgtttatgatagcctgcgtaaagccggtgcaagtgatgcaggttgggttctgaataccgatagcatgcatagctggctggaaaaaaatggctttaaactgattgcccagaacaaagaatggtcagcaaaacgtggtgatgtggtgatttttggtaaaaaaggtgcaagcggtggtagcgcaggtcatgttgttatctttattagcagcacccagattattcactgtacctggaaaagcgcaaccgcaaatggtgtttatgttgataatgaagcaaccacctgtccgtatagcatgggttggtatgtttatcgtctgaatggtggtagcacccctccg

SEQ ID NO: 96 - DNA, 195 bp, Artificial sequence
  Encoding SEQ ID NO:3
gaggccacctttattaacggcaatgcaccgattaccacccgtaaaaacaaaccgagcctgagcagccagaccgcaacaccgctgtatccgggtcagagcgttcgttatctgggctggaaatcagcagaaggttatatttggatttatgccaccgatggtcgttatattccggttcgtccggttggtaaagaagca

SEQ ID NO: 97 - DNA, 939 bp, Artificial sequence
  encoding enterococcal phage phi1 endolysin w/o initial methionine
agcaacatcaatatggaaaccgccattgcaaatatgtatgcactgaaagcacgtggcattacctatagcatgaattatagccgtaccggtgcagatggcaccggtgattgtagcggcaccgtttatgatagcctgcgtaaagccggtgcaagtgatgcaggttgggttctgaataccgatagcatgcatagctggctggaaaaaaatggctttaaactgattgcccagaacaaagaatggtcagcaaaacgtggtgatgtggtgatttttggtaaaaaaggtgcaagcggtggtagcgcaggtcatgttgttatctttattagcagcacccagattattcactgtacctggaaaagcgcaaccgcaaatggtgtttatgttgataatgaagcaaccacctgtccgtatagcatgggttggtatgtttatcgtctgaatggtggtagcacccctccgaaaccgaataccaaaaaagttaaagttctgaaacacgccaccaattggagcccgagcagcaaaggtgccaaaatggcaagctttgttaaaggtggtacgtttgaagttaaacagcagcgtccgattagctacagctatagcaatcaagaatatctgatcgtgaataaaggcaccgttctgggttgggtgctgagccaggatattgaaggtggttatggtagcgatcgtgttggtggtagtaaaccgaaactgcctgcaggttttacaaaagaagaggccacctttattaacggcaatgcaccgattaccacccgtaaaaacaaaccgagcctgagcagccagaccgcaacaccgctgtatccgggtcagagcgttcgttatctgggctggaaatcagcagaaggttatatttggatttatgccaccgatggtcgttatattccggttcgtccggttggtaaagaagcatggggcacctttaaa

SEQ ID NO: 98 - DNA, 63 bp, Artificial sequence
  encoding Buforin II vertebrate
acccgtagctctcgtgctggcctgcagtttccggttggtcgcgtgcaccgtctgctccgcaaa

SEQ ID NO: 99 - DNA, 1011 bp, artificial sequence
  Encoding enterococcal bacteriophae phi1 endolysin plus Buforin II
atgacccgtagctctcgtgctggcctgcagtttccggttggtcgcgtgcaccgtctgctccgcaaaggatccagcaacatcaatatggaaaccgccattgcaaatatgtatgcactgaaagcacgtggcattacctatagcatgaattatagccgtaccggtgcagatggcaccggtgattgtagcggcaccgtttatgatagcctgcgtaaagccggtgcaagtgatgcaggttgggttctgaataccgatagcatgcatagctggctggaaaaaaatggctttaaactgattgcccagaacaaagaatggtcagcaaaacgtggtgatgtggtgatttttggtaaaaaaggtgcaagcggtggtagcgcaggtcatgttgttatctttattagcagcacccagattattcactgtacctggaaaagcgcaaccgcaaatggtgtttatgttgataatgaagcaaccacctgtccgtatagcatgggttggtatgtttatcgtctgaatggtggtagcacccctccgaaaccgaataccaaaaaagttaaagttctgaaacacgccaccaattggagcccgagcagcaaaggtgccaaaatggcaagctttgttaaaggtggtacgtttgaagttaaacagcagcgtccgattagctacagctatagcaatcaagaatatctgatcgtgaataaaggcaccgttctgggttgggtgctgagccaggatattgaaggtggttatggtagcgatcgtgttggtggtagtaaaccgaaactgcctgcaggttttacaaaagaagaggccacctttattaacggcaatgcaccgattaccacccgtaaaaacaaaccgagcctgagcagccagaccgcaacaccgctgtatccgggtcagagcgttcgttatctgggctggaaatcagcagaaggttatatttggatttatgccaccgatggtcgttatattccggttcgtccggttggtaaagaagcatggggcacctttaaa

SEQ ID NO: 100 - protein, 7 aa, Homo sapiens
HPQYNQR

SEQ ID NO: 101 - protein, 322 aa, Artificial sequence
  Enterococcal bacteriophae phi1 endolysin plus peptide, w/o starting methionine
SNINMETAIANMYALKARGITYSMNYSRTGADGTGDCSGTVYDSLRKAGASDAGWVLNTDSMHSWLEKNGFKLIAQNKEWSAKRGDVVIFGKKGASGGSAGHVVIFISSTQIIHCTWKSATANGVYVDNEATTCPYSMGWYVYRLNGGSTPPKPNTKKVKVLKHATNWSPSSKGAKMASFVKGGTFEVKQQRPISYSYSNQEYLIVNKGTVLGWVLSQDIEGGYGSDRVGGSKPKLPAGFTKEEATFINGNAPITTRKNKPSLSSQTATPLYPGQSVRYLGWKSAEGYIWIYATDGRYIPVRPVGKEAWGTFKGSHPQYNQR

SEQ ID NO: 102 - protein, 323 aa, Artificial sequence
  Enterococcal bacteriophae phi1 endolysin plus peptide
MSNINMETAIANMYALKARGITYSMNYSRTGADGTGDCSGTVYDSLRKAGASDAGWVLNTDSMHSWLEKNGFKLIAQNKEWSAKRGDVVIFGKKGASGGSAGHVVIFISSTQIIHCTWKSATANGVYVDNEATTCPYSMGWYVYRLNGGSTPPKPNTKKVKVLKHATNWSPSSKGAKMASFVKGGTFEVKQQRPISYSYSNQEYLIVNKGTVLGWVLSQDIEGGYGSDRVGGSKPKLPAGFTKEEATFINGNAPITTRKNKPSLSSQTATPLYPGQSVRYLGWKSAEGYIWIYATDGRYIPVRPVGKEAWGTFKGSHPQYNQR

SEQ ID NO: 103 - protein, 329 aa, Artificial sequence
  Enterococcal bacteriophae phi1 endolysin plus HisTag and peptide
MSNINMETAIANMYALKARGITYSMNYSRTGADGTGDCSGTVYDSLRKAGASDAGWVLNTDSMHSWLEKNGFKLIAQNKEWSAKRGDVVIFGKKGASGGSAGHVVIFISSTQIIHCTWKSATANGVYVDNEATTCPYSMGWYVYRLNGGSTPPKPNTKKVKVLKHATNWSPSSKGAKMASFVKGGTFEVKQQRPISYSYSNQEYLIVNKGTVLGWVLSQDIEGGYGSDRVGGSKPKLPAGFTKEEATFINGNAPITTRKNKPSLSSQTATPLYPGQSVRYLGWKSAEGYIWIYATDGRYIPVRPVGKEAWGTFKGSHHHHHHHPQYNQR

SEQ ID NO: 104 - protein, 241 aa, Artificial Sequence
  aa 2-242 of Streptococcus suis enzyme (WP_029171101.1); C136S
GVNIETALRWMSDRKGRVTYSMDYRNGPNSFDCSSSVYYALMSAGAISAGWAVNTEYEHDWLLKNGYKLIAENTDWDAKRGDIFIWGRRGQSAGAGGHTGIFIDPDNIIHCNYARNSITVDNYNQTAAASGWMYSYVYRLANQTSTAGKSLETLVQETLAGKYGNGDQRKAALGNQYEAVMAVINGKATAPKKTVDQLAQEVIAGKHGNGEARKQSLGADYPAVQKRVTELLKKQPSEPSK

SEQ ID NO: 105 - protein, 346 aa, Artificial sequence
  aa 2-242 of Streptococcus suis enzyme (WP_029171101.1); C136S, plus enterococcal bacteriophae phi1 endolysin CBD plus HisTag and peptide
MGVNIETALRWMSDRKGRVTYSMDYRNGPNSFDCSSSVYYALMSAGAISAGWAVNTEYEHDWLLKNGYKLIAENTDWDAKRGDIFIWGRRGQSAGAGGHTGIFIDPDNIIHCNYARNSITVDNYNQTAAASGWMYSYVYRLANQTSTAGKSLETLVQETLAGKYGNGDQRKAALGNQYEAVMAVINGKATAPKKTVDQLAQEVIAGKHGNGEARKQSLGADYPAVQKRVTELLKKQPSEPSKGSDRVGGSKPKLPAGFTKEEATFINGNAPITTRKNKPSLSSQTATPLYPGQSVRYLGWKSAEGYIWIYATDGRYIPVRPVGKEAWGTFKGSHHHHHHHPQYNQR